European Patent Application EP 4 428 152 A1, published September 11, 2024. Title: MONOCLONAL ANTIBODY AGAINST HLA-G1, HLA-G4 AND HLA-G5 ISOFORMS AND USE THEREOF. Applicant: TAIZHOU ENZE MEDICAL CENTER (GROUP). The sequence listing filed with the application follows.

SEQUENCE LISTING (17 sequences)

SEQ ID NO: 1 - protein, 123 aa, (Hybridoma)（YWHG-4)
GDIVITQDELSLPVSLGDQAAISCRSSQSIVHSNGNTYLEWYLQKPGQSPKLLIYKVSNRFSGVPDRFRGSGSGTDFTLKISRVEAEDLGVYYCFQASHVPYTFGGGTKLEIKRADAAPTGSI

SEQ ID NO: 2 - protein, 11 aa, (Hybridoma)（YWHG-4)
QSIVHSNGNTY

SEQ ID NO: 3 - protein, 3 aa, (Hybridoma)（YWHG-4)
KVS

SEQ ID NO: 4 - protein, 9 aa, (Hybridoma)（YWHG-4)
FQASHVPYT

SEQ ID NO: 5 - protein, 131 aa, (Hybridoma)（YWHG-4)
VQLQQSGAEVVRPGTSVKVSCKASGYASTNYLVEWIKQRPGQGLEWIGVINPGSGRIYYSEKFKGKTTLTADKSSSNAYMQLSSLTSDDSAVYFCARHYGNSAWFAYWGQGTLVTVSAAKTTPKLVYPLAP

SEQ ID NO: 6 - protein, 8 aa, (Hybridoma)（YWHG-4)
GYASTNYL

SEQ ID NO: 7 - protein, 8 aa, (Hybridoma)（YWHG-4)
INPGSGRI

SEQ ID NO: 8 - protein, 12 aa, (Hybridoma)（YWHG-4)
ARHYGNSAWFAY

SEQ ID NO: 9 - protein, 26 aa, (Hybridoma)（YWHG-4)
GDIVITQDELSLPVSLGDQAAISCRS

SEQ ID NO: 10 - protein, 17 aa, (Hybridoma)（YWHG-4)
LEWYLQKPGQSPKLLIY

SEQ ID NO: 11 - protein, 36 aa, (Hybridoma)（YWHG-4)
NRFSGVPDRFRGSGSGTDFTLKISRVEAEDLGVYYC

SEQ ID NO: 12 - protein, 24 aa, (Hybridoma)（YWHG-4)
VQLQQSGAEVVRPGTSVKVSCKAS

SEQ ID NO: 13 - protein, 17 aa, (Hybridoma)（YWHG-4)
VEWIKQRPGQGLEWIGV

SEQ ID NO: 14 - protein, 38 aa, (Hybridoma)（YWHG-4)
YYSEKFKGKTTLTADKSSSNAYMQLSSLTSDDSAVYFC

SEQ ID NO: 15 - DNA, 369 bp, (Hybridoma)（YWHG-4)
ggtgatatcgtgataacccaagatgaactctccctgcctgtcagtcttggagatcaagccgccatctcttgcagatctagtcagagcattgtacatagtaatggaaacacctatttagaatggtatttgcagaaaccaggccagtctccaaagctcctgatctacaaagtttccaaccgattttctggggtcccagacaggttcagaggcagtggatcagggacagattttacactcaagatcagcagagtggaggctgaggatctgggagtttattactgctttcaagcttcacatgttccgtacacgttcggaggggggaccaagctggaaataaaacgggctgatgctgcaccaactggatccatc

SEQ ID NO: 16 - DNA, 393 bp, (Hybridoma)（YWHG-4)
gtccaactgcagcagtcaggagctgaggtggtaaggcctgggacttcagtgaaggtgtcctgcaaggcttctggatacgcctccactaattacttagtagagtggataaagcagaggcctggacagggccttgagtggattggagtgattaatcctggaagtggacgtatttactacagtgagaagttcaagggcaagacaacactgactgcagacaaatcctccagcaatgcctacatgcagctcagcagccttacatctgatgactctgcggtttatttctgtgcaagacactatggtaactccgcctggtttgcttactggggccaagggactctggtcactgtctctgcagccaaaacgacacccaagcttgtctatccactggcccct

SEQ ID NO: 17 - protein, 20 aa, (Hybridoma)（YWHG-4)
RGYYNQSEASSHTLQWMIGC